European Patent Application EP 4 643 873 A2, published November 5, 2025. Title: DPEP-1 Binding Compositions and Methods of Use. Applicant: Arch Biopartners, Inc. The sequence listing filed with the application follows.

SEQUENCE LISTING (36 sequences)

SEQ ID NO: 1 - protein, 16 aa, Homo sapiens
LSALTPSPSWLKYKAL

SEQ ID NO: 2 - protein, 13 aa, Homo sapiens
CGFECVRQCPERC

SEQ ID NO: 3 - protein, 8 aa, Homo sapiens
CGFELETC

SEQ ID NO: 4 - protein, 17 aa, Homo sapiens
  SITE 1: note = MISC_FEATURE - X is any naturally-occurring amino acid, unconventional amino acid or amino acid analog
XLSALTPSPSWLKYKAL

SEQ ID NO: 5 - protein, 18 aa, Homo sapiens
  REGION 1..2: note = MISC_FEATURE - X is any naturally-occurring amino acid, unconventional amino acid or amino acid analog
XXLSALTPSPSWLKYKAL

SEQ ID NO: 6 - protein, 19 aa, Homo sapiens
  REGION 1..3: note = MISC_FEATURE - X is any naturally-occurring amino acid, unconventional amino acid or amino acid analog
XXXLSALTPSPSWLKYKAL

SEQ ID NO: 7 - protein, 20 aa, Homo sapiens
  REGION 1..4: note = MISC_FEATURE - X is any naturally-occurring amino acid, unconventional amino acid or amino acid analog
XXXXLSALTPSPSWLKYKAL

SEQ ID NO: 8 - protein, 17 aa, Homo sapiens
  SITE 1: note = MISC_FEATURE - X is any naturally-occurring amino acid, unconventional amino acid or amino acid analog
  SITE 17: note = misc_feature - Xaa can be any naturally occurring amino acid
LSALTPSPSWLKYKALX

SEQ ID NO: 9 - protein, 18 aa, Homo sapiens
  REGION 1..2: note = MISC_FEATURE - X is any naturally-occurring amino acid, unconventional amino acid or amino acid analog
  REGION 17..18: note = misc_feature - Xaa can be any naturally occurring amino acid
LSALTPSPSWLKYKALXX

SEQ ID NO: 10 - protein, 19 aa, Homo sapiens
  REGION 17..19: note = misc_feature - Xaa can be any naturally occurring amino acid
LSALTPSPSWLKYKALXXX

SEQ ID NO: 11 - protein, 20 aa, Homo sapiens
  REGION 1..3: note = MISC_FEATURE - X is any naturally-occurring amino acid, unconventional amino acid or amino acid analog
  REGION 17..20: note = misc_feature - Xaa can be any naturally occurring amino acid
LSALTPSPSWLKYKALXXXX

SEQ ID NO: 12 - protein, 18 aa, Homo sapiens
  SITE 1: note = MISC_FEATURE - X is any naturally-occurring amino acid, unconventional amino acid or amino acid analog
  SITE 18: note = MISC_FEATURE - X is any naturally-occurring amino acid, unconventional amino acid or amino acid analog
XLSALTPSPSWLKYKALX

SEQ ID NO: 13 - protein, 19 aa, Homo sapiens
  SITE 1: note = MISC_FEATURE - X is any naturally-occurring amino acid, unconventional amino acid or amino acid analog
  REGION 18..19: note = MISC_FEATURE - X is any naturally-occurring amino acid, unconventional amino acid or amino acid analog
XLSALTPSPSWLKYKALXX

SEQ ID NO: 14 - protein, 20 aa, Homo sapiens
  SITE 1: note = MISC_FEATURE - X is any naturally-occurring amino acid, unconventional amino acid or amino acid analog
  REGION 18..20: note = MISC_FEATURE - X is any naturally-occurring amino acid, unconventional amino acid or amino acid analog
XLSALTPSPSWLKYKALXXX

SEQ ID NO: 15 - protein, 21 aa, Homo sapiens
  SITE 1: note = MISC_FEATURE - X is any naturally-occurring amino acid, unconventional amino acid or amino acid analog
  REGION 18..21: note = MISC_FEATURE - X is any naturally-occurring amino acid, unconventional amino acid or amino acid analog
XLSALTPSPSWLKYKALXXXX

SEQ ID NO: 16 - protein, 22 aa, Homo sapiens
  SITE 1: note = MISC_FEATURE - X is any naturally-occurring amino acid, unconventional amino acid or amino acid analog
  REGION 18..22: note = MISC_FEATURE - X is any naturally-occurring amino acid, unconventional amino acid or amino acid analog
XLSALTPSPSWLKYKALXXXXX

SEQ ID NO: 17 - protein, 19 aa, Homo sapiens
  REGION 1..2: note = MISC_FEATURE - X is any naturally-occurring amino acid, unconventional amino acid or amino acid analog
  SITE 19: note = MISC_FEATURE - X is any naturally-occurring amino acid, unconventional amino acid or amino acid analog
XXLSALTPSPSWLKYKALX

SEQ ID NO: 18 - protein, 19 aa, Homo sapiens
  REGION 1..2: note = MISC_FEATURE - X is any naturally-occurring amino acid, unconventional amino acid or amino acid analog
  REGION 18..19: note = MISC_FEATURE - X is any naturally-occurring amino acid, unconventional amino acid or amino acid analog
XXLSALTPSPSWLKYKAXX

SEQ ID NO: 19 - protein, 21 aa, Homo sapiens
  REGION 1..2: note = MISC_FEATURE - X is any naturally-occurring amino acid, unconventional amino acid or amino acid analog
  REGION 19..20: note = MISC_FEATURE - X is any naturally-occurring amino acid, unconventional amino acid or amino acid analog
  SITE 21: note = misc_feature - Xaa can be any naturally occurring amino acid
XXLSALTPSPSWLKYKALXXX

SEQ ID NO: 20 - protein, 22 aa, Homo sapiens
  REGION 1..2: note = MISC_FEATURE - X is any naturally-occurring amino acid, unconventional amino acid or amino acid analog
  REGION 19..22: note = MISC_FEATURE - X is any naturally-occurring amino acid, unconventional amino acid or amino acid analog
XXLSALTPSPSWLKYKALXXXX

SEQ ID NO: 21 - protein, 23 aa, Homo sapiens
  REGION 1..2: note = MISC_FEATURE - X is any naturally-occurring amino acid, unconventional amino acid or amino acid analog
  REGION 19..23: note = MISC_FEATURE - X is any naturally-occurring amino acid, unconventional amino acid or amino acid analog
XXLSALTPSPSWLKYKALXXXXX

SEQ ID NO: 22 - protein, 20 aa, Homo sapiens
  REGION 1..3: note = MISC_FEATURE - X is any naturally-occurring amino acid, unconventional amino acid or amino acid analog
  SITE 20: note = MISC_FEATURE - X is any naturally-occurring amino acid, unconventional amino acid or amino acid analog
XXXLSALTPSPSWLKYKALX

SEQ ID NO: 23 - protein, 21 aa, Homo sapiens
  REGION 1..3: note = MISC_FEATURE - X is any naturally-occurring amino acid, unconventional amino acid or amino acid analog
  REGION 20..21: note = MISC_FEATURE - X is any naturally-occurring amino acid, unconventional amino acid or amino acid analog
XXXLSALTPSPSWLKYKALXX

SEQ ID NO: 24 - protein, 22 aa, Homo sapiens
  REGION 1..3: note = MISC_FEATURE - X is any naturally-occurring amino acid, unconventional amino acid or amino acid analog
  REGION 20..22: note = MISC_FEATURE - X is any naturally-occurring amino acid, unconventional amino acid or amino acid analog
XXXLSALTPSPSWLKYKALXXX

SEQ ID NO: 25 - protein, 23 aa, Homo sapiens
  REGION 1..3: note = MISC_FEATURE - X is any naturally-occurring amino acid, unconventional amino acid or amino acid analog
  REGION 20..23: note = MISC_FEATURE - X is any naturally-occurring amino acid, unconventional amino acid or amino acid analog
XXXLSALTPSPSWLKYKALXXXX

SEQ ID NO: 26 - protein, 24 aa, Homo sapiens
  REGION 1..3: note = MISC_FEATURE - X is any naturally-occurring amino acid, unconventional amino acid or amino acid analog
  REGION 20..24: note = MISC_FEATURE - X is any naturally-occurring amino acid, unconventional amino acid or amino acid analog
XXXLSALTPSPSWLKYKALXXXXX

SEQ ID NO: 27 - protein, 21 aa, Homo sapiens
  REGION 1..4: note = MISC_FEATURE - X is any naturally-occurring amino acid, unconventional amino acid or amino acid analog
  SITE 21: note = MISC_FEATURE - X is any naturally-occurring amino acid, unconventional amino acid or amino acid analog
XXXXLSALTPSPSWLKYKALX

SEQ ID NO: 28 - protein, 22 aa, Homo sapiens
  REGION 1..4: note = MISC_FEATURE - X is any naturally-occurring amino acid, unconventional amino acid or amino acid analog
  REGION 21..22: note = MISC_FEATURE - X is any naturally-occurring amino acid, unconventional amino acid or amino acid analog
XXXXLSALTPSPSWLKYKALXX

SEQ ID NO: 29 - protein, 23 aa, Homo sapiens
  REGION 1..4: note = MISC_FEATURE - X is any naturally-occurring amino acid, unconventional amino acid or amino acid analog
  REGION 21..23: note = MISC_FEATURE - X is any naturally-occurring amino acid, unconventional amino acid or amino acid analog
XXXXLSALTPSPSWLKYKALXXX

SEQ ID NO: 30 - protein, 24 aa, Homo sapiens
  REGION 1..4: note = MISC_FEATURE - X is any naturally-occurring amino acid, unconventional amino acid or amino acid analog
  REGION 21..24: note = MISC_FEATURE - X is any naturally-occurring amino acid, unconventional amino acid or amino acid analog
XXXXLSALTPSPSWLKYKALXXXX

SEQ ID NO: 31 - protein, 25 aa, Homo sapiens
  REGION 1..4: note = MISC_FEATURE - X is any naturally-occurring amino acid, unconventional amino acid or amino acid analog
  REGION 21..25: note = MISC_FEATURE - X is any naturally-occurring amino acid, unconventional amino acid or amino acid analog
XXXXLSALTPSPSWLKYKALXXXXX

SEQ ID NO: 32 - protein, 22 aa, Homo sapiens
  REGION 1..5: note = MISC_FEATURE - X is any naturally-occurring amino acid, unconventional amino acid or amino acid analog
  SITE 22: note = MISC_FEATURE - X is any naturally-occurring amino acid, unconventional amino acid or amino acid analog
XXXXXLSALTPSPSWLKYKALX

SEQ ID NO: 33 - protein, 23 aa, Homo sapiens
  REGION 1..5: note = MISC_FEATURE - X is any naturally-occurring amino acid, unconventional amino acid or amino acid analog
  REGION 22..23: note = MISC_FEATURE - X is any naturally-occurring amino acid, unconventional amino acid or amino acid analog
XXXXXLSALTPSPSWLKYKALXX

SEQ ID NO: 34 - protein, 24 aa, Homo sapiens
  REGION 1..5: note = MISC_FEATURE - X is any naturally-occurring amino acid, unconventional amino acid or amino acid analog
  REGION 22..24: note = MISC_FEATURE - X is any naturally-occurring amino acid, unconventional amino acid or amino acid analog
XXXXXLSALTPSPSWLKYKALXXX

SEQ ID NO: 35 - protein, 25 aa, Homo sapiens
  REGION 1..5: note = MISC_FEATURE - X is any naturally-occurring amino acid, unconventional amino acid or amino acid analog
  REGION 22..25: note = MISC_FEATURE - X is any naturally-occurring amino acid, unconventional amino acid or amino acid analog
XXXXXLSALTPSPSWLKYKALXXXX

SEQ ID NO: 36 - protein, 26 aa, Homo sapiens
  REGION 1..5: note = MISC_FEATURE - X is any naturally-occurring amino acid, unconventional amino acid or amino acid analog
  REGION 22..26: note = MISC_FEATURE - X is any naturally-occurring amino acid, unconventional amino acid or amino acid analog
XXXXXLSALTPSPSWLKYKALXXXXX